European Patent Application EP 4 763 860 A1, published June 24, 2026. Title: Method for VHH library construction. Applicant: Biotalys NV. Application EP. The sequence listing filed with the application follows.

SEQUENCE LISTING (18 sequences)

SEQ ID NO: 1 - DNA, 24 bp, synthetic construct
  source 1..24: mol_type = other DNA
gcaagaccttcatctgcaacgtag

SEQ ID NO: 2 - DNA, 20 bp, synthetic construct
  source 1..20: mol_type = other DNA
ttgtccaccttggtgctgct

SEQ ID NO: 3 - DNA, 21 bp, synthetic construct
  source 1..21: mol_type = other DNA
ggctgagctgggtggtcctgg

SEQ ID NO: 4 - DNA, 21 bp, synthetic construct
  source 1..21: mol_type = other DNA
ggctgagtttggtggtcctgg

SEQ ID NO: 5 - DNA, 23 bp, synthetic construct
  source 1..23: mol_type = other DNA
ggtacgtgctgttgaactgttcc

SEQ ID NO: 6 - DNA, 292 bp, Vicugna pacos
  source 1..292: mol_type = other DNA
tccaccaaggccccatcggtctatcctctgactgctagatgcggggacacgcctggctccacagtggccttcggctgcctggtctggggctacatccctgagccggtgacggtgacttggaactcaggcgccctgtccagcggcgtccacaccttcccatcagtcttcatgtcctcggggctctactccctcagcagcttggtgacactgcccacaagcagctcaaccggcaagaccttcatctgcaacgtagcccacccggccagcagcaccaaggtggacaagcgtgtgg

SEQ ID NO: 7 - DNA, 292 bp, Lama glama; identical to SEQ ID NO: 6
  source 1..292: mol_type = other DNA

SEQ ID NO: 8 - DNA, 292 bp, Vicugna pacos
  source 1..292: mol_type = other DNA
tccaccaaggccccatcggtctatcctctgactgctagatgcggggacacgcctggctccacagtggccttcggctgcctagtctggggctatatccctgagccggtgacggtgacgtggaactcgggcgccctgtccagcggcgtccacaccttcccatcagtcttcatgtcctcggggctctacaccctcagcagcttggtgaccatgcccgccagcagctcgaccggcaagaccttcatctgcaacgtagcccacccggccagcagcaccaaggtggacaagcgtgtgg

SEQ ID NO: 9 - DNA, 292 bp, Camelus dromedarius
  source 1..292: mol_type = other DNA
tccaccaaggccccatcggtctatcctctgactgctagatgcggggacacgcctggctccacggtggccttcggctgcctggtctggggctacatccctgagccggtgacggtgacctggaactcgggcgccctgtccagcggcatccacaccttcccatctgttctcatgtcctcggggctctactcactcagcagcttagtgactctgcccgccagcagctcgtccggcaagaacttcatctgcaacgtagcccacccggccagcagcactaaggtggacaagcgtgtgg

SEQ ID NO: 10 - DNA, 292 bp, Camelus dromedarius
  source 1..292: mol_type = other DNA
tccaccaaggccccatcggtctatcctctgactgctagatggggggacacgcctggctccacggtggccttcggctgcctggtgtggggctacatccctgagccagtgacagtgacctggaactcgggtgccctgtccagcggcgtccacaccttcccgtcagtcttcatgtcctcggggctctacaccctcagcagcttagtgactctgcccaccagcagctcgaccggcaagaccttcttctgcaacgtagcccacccggccagcagcaccaaggtggacaagcgtgtgg

SEQ ID NO: 11 - DNA, 292 bp, Camelus dromedarius
  source 1..292: mol_type = other DNA
tccaccaaggccccatcggtctatcctctgactgctagatccggggatacgcctggctccacggtggccttcggctgcctggtctggggctacatccctgagccggtgacggtgacctggaattcaggcgctgtgtccagcggcatccacaccttcccatctgttctcatgtccttggggctctactcactcagcagcttagtgactctgcccaccagcacctcgaccggaaagaccttcatctccaacgtagcccacccagccagcagcaccaaggtggacaagagtgtgg

SEQ ID NO: 12 - DNA, 292 bp, Camelus bactrianus; identical to SEQ ID NO: 9
  source 1..292: mol_type = other DNA

SEQ ID NO: 13 - DNA, 292 bp, Camelus bactrianus
  source 1..292: mol_type = other DNA
tccaccaaggccccatcggtctatcctctgactgctagatgcggggacacgcctggctccacggtggccttcggctgcctggtctggggctacatccctgagccggtgacggtgacctggaactcgggtgccctgtccagcggcgtccacaccttcccgtcagtcttcatgtcctcggggctctacaccctcagcagcttagtgactctgcccaccagcagctcgaccggcaagaccttcttctgcaacgtagcccacccggccagcagcaccaaggtggacaagcgtgtgg

SEQ ID NO: 14 - DNA, 292 bp, Camelus bactrianus
  source 1..292: mol_type = other DNA
tccaccaaggccccatcggtctatcctccgactgctggatgctgggacatgcctgactccacggtggccttcggctgcctggtctggggctacatccctgagccggtgacggtgacctggaactcgggcgccctgtccagcggcatccacaccttcccgtccattctcatgtccttgggtctctactccctcagcagcttggcgaccatgcccgccagcagctcggccggcaagaccttcatctgcaacgtagcccacccggccagcagcaccaaggcggacaagcgtgtgg

SEQ ID NO: 15 - DNA, 292 bp, Camelus bactrianus
  source 1..292: mol_type = other DNA
tccaccaaggccccatcggtctatcctccgactgctggatgcggggacgctcctggctccacggtgcccttcggctgcctggtctggggctacatccctgagccggtgacggtgacctggaactcgggcgccctgtccagcggcatccacaccttcccgtccattctcatgtcctcggggctctactccctcagcagcttggcgaccatgcccgccagcagctcggccggcaagaccttcatctgcaacgtagcccacccggtcagcagcaccaaggcggacaagcatgtgg

SEQ ID NO: 16 - DNA, 35 bp, synthetic construct
  source 1..35: mol_type = other DNA
tgatgctcttccgctgaggagacggtgacctgggt

SEQ ID NO: 17 - DNA, 38 bp, synthetic construct
  source 1..38: mol_type = other DNA
cttggctcttctgtgcagctgcaggagtctgggggagg

SEQ ID NO: 18 - DNA, 4545 bp, synthetic construct
  source 1..4545: mol_type = other DNA
tttacggttcctggccttttgctggccttttgctcacatgttctttcctgcgttatcccctgattctgtggataaccgtattaccgcctttgagtgagctgataccgctcgccgcagccgaacgaccgagcgcagcgagtcagtgagcgaggaagcggaggagcgcccaatacgcaaaccgcctctccccgcgcgttggccgattcattaatgcagctggcacgacaggtttcccgactggaaagcgggcagtgagcgcaacgcaattaatgtgagttagctcactcattaggcaccccaggctttacactttatgcttccggctcgtatgttgtgtggaattgtgagcggataacaatttcacaagcttaaggagacagtacatatgaaatacctattgcctacggcagccgctggattgttattactcgcggcccagccggccatggccgacgtgcgaagagcgaggcatgatccgctcttcgagttgatcgtacgtagctcgaggagccgatcagctcttccagcggccgcagactacaaagaccatgacggtgattataaagatcatgacatcgattacaaggatgacgatgacaaggccgcatagactgttgaaagttgtttagcaaaacctcatacagaaaattcatttactaacgtctggaaagacgacaaaactttagatcgttacgctaactatgagggctgtctgtggaatgctacaggcgttgtggtttgtactggtgacgaaactcagtgttacggtacatgggttcctattgggcttgctatccctgaaaatgagggtggtggctctgagggtggcggttctgagggtggcggttctgagggtggcggtactaaacctcctgagtacggtgatacacctattccgggctatacttatatcaaccctctcgacggcacttatccgcctggtactgagcaaaaccccgctaatcctaatccttctcttgaggagtctcagcctcttaatactttcatgtttcagaataataggttccgaaataggcagggtgcattaactgtttatacgggcactgttactcaaggcactgaccccgttaaaacttattaccagtacactcctgtatcatcaaaagccatgtatgacgcttactggaacggtaaattcagagactgcgctttccattctggctttaatgaggatccattcgtttgtgaatatcaaggccaatcgtctgacctgcctcaacctcctgtcaatgctggcggcggctctggtggtggttctggtggcggctctgagggtggcggctctgagggtggcggttctgagggtggcggctctgagggtggcggttccggtggcggctccggttccggtgattttgattatgaaaaaatggcaaacgctaataagggggctatgaccgaaaatgccgatgaaaacgcgctacagtctgacgctaaaggcaaacttgattctgtcgctactgattacggtgctgctatcgatggtttcattggtgacgtttccggccttgctaatggtaatggtgctactggtgattttgctggctctaattcccaaatggctcaagtcggtgacggtgataattcacctttaatgaataatttccgtcaatatttaccttctttgcctcagtcggttgaatgtcgcccttatgtctttggcgctggtaaaccatatgaattttctattgattgtgacaaaataaacttattccgtggtgtctttgcgtttcttttatatgttgccacctttatgtatgtattttcgacgtttgctaacatactgcgtaataaggagtcttaataagaattcactggccgtcgttttacaacgtcgtgactgggaaaaccctggcgttacccaacttaatcgccttgcagcacatccccctttcgccagctggcgtaatagcgaagaggcccgcaccgatcgcccttcccaacagttgcgcagcctgaatggcgaatggcgcctgatgcggtattttctccttacgcatctgtgcggtatttcacaccgcatacgtcaaagcaaccatagtacgcgccctgtagcggcgcattaagcgcggcgggtgtggtggttacgcgcagcgtgaccgctacacttgccagcgccttagcgcccgctcctttcgctttcttcccttcctttctcgccacgttcgccggctttccccgtcaagctctaaatcgggggctccctttagggttccgatttagtgctttacggcacctcgaccccaaaaaacttgatttgggtgatggttcacgtagtgggccatcgccctgatagacggtttttcgccctttgacgttggagtccacgttctttaatagtggactcttgttccaaactggaacaacactcaactctatctcgggctattcttttgatttataagggattttgccgatttcggtctattggttaaaaaatgagctgatttaacaaaaatttaacgcgaattttaacaaaatattaacgtttacaattttatggtgcactctcagtacaatctgctctgatgccgcatagttaagccagccccgacacccgccaacacccgctgacgcgccctgacgggcttgtctgctcccggcatccacttacagacaagctgtgaccgtctccgggagctgcatgtgtcagaggttttcaccgtcatcaccgaaacgcgcgagacgaaagggcctcgtgatacgcctatttttataggttaatgtcatgataataatggtttcttagacgtcaggtggcacttttcggggaaatgtgcgcggaacccctatttgtttatttttctaaatacattcaaatatgtatccgctcatgagacaataaccctgataaatgcttcaataatattgaaaaaggaagagtatgagtattcaacatttccgtgtcgcccttattcccttttttgcggcattttgccttcctgtttttgctcacccagaaacgctggtgaaagtaaaagatgctgaagatcagttgggtgcacgagtgggttacatcgaactggatctcaacagcggtaagatccttgagagttttcgccccgaagaacgttttccaatgatgagcacttttaaagttctgctatgtggcgcggtattatcccgtattgacgccgggcaagagcaactcggtcgccgcatacactattctcagaatgacttggttgagtactcaccagtcacagaaaagcatcttacggatggcatgacagtaagagaattatgcagtgctgccataaccatgagtgataacactgcggccaacttacttctgacaacgatcggaggaccgaaggagctaaccgcttttttgcacaacatgggggatcatgtaactcgccttgatcgttgggaaccggagctgaatgaagccataccaaacgacgagcgtgacaccacgatgcctgtagcaatggcaacaacgttgcgcaaactattaactggcgaactacttactctagcttcccggcaacaattaatagactggatggaggcggataaagttgcaggaccacttctgcgctcggcccttccggctggctggtttattgctgataaatctggagccggtgagcgtgggtctcgcggtatcattgcagcactggggccagatggtaagccctcccgtatcgtagttatctacacgacggggagtcaggcaactatggatgaacgaaatagacagatcgctgagataggtgcctcactgattaagcattggtaactgtcagaccaagtttactcatatatactttagattgatttaaaacttcatttttaatttaaaaggatctaggtgaagatcctttttgataatctcatgaccaaaatcccttaacgtgagttttcgttccactgagcgtcagaccccgtagaaaagatcaaaggatcttcttgagatcctttttttctgcgcgtaatctgctgcttgcaaacaaaaaaaccaccgctaccagcggtggtttgtttgccggatcaagagctaccaactctttttccgaaggtaactggcttcagcagagcgcagataccaaatactgttcttctagtgtagccgtagttaggccactacttcaagaactctgtagcaccgcctacatacctcgctctgctaatcctgttaccagtggctgctgccagtggcgataagtcgtgtcttaccgggttggactcaagacgatagttaccggataaggcgcagcggtcgggctgaacggggggttcgtgcacacagcccagcttggagcgaacgacctacaccgaactgagatacctacagcgtgagctatgagaaagcgccacgcttcccgaagggagaaaggcggacaggtatccggtaagcggcagggtcggaacaggagagcgcacgagggagcttccagggggaaacgcctggtatctttatagtcctgtcgggtttcgccacctctgacttgagcgtcgatttttgtgatgctcgtcaggggggcggagcctatggaaaaacgccagcaacgcggcctt